European Patent Specification EP 3 033 437 B1, published November 8, 2023. Title: COMPOSITIONS AND METHODS FOR DETECTING HEV NUCLEIC ACID. Applicant: Gen-Probe Incorporated GAO, Kui ONG, Edgar O. COLE, Jennifer. The sequence listing filed with the application follows.

SEQUENCE LISTING (79 sequences)

SEQ ID NO: 1 - DNA, 7256 bp, Hepatitis E virus
  ref <308>: AB074918.2 GI:21218075
  ref <309>: 2008-12-17
  ref <313>: (1)..(7256)
gcagaccacgtatgtggtcgatgccatggaggcccatcagttcattaaggctcctggcattactactgccattgagcaggctgctctggctgcggccaattccgccttggcgaatgctgtggtggtccggccgttcttatctcgtgtacaaactgagattcttattaatttgatgcaaccccggcagttggttttccgccctgaggtgctctggaatcaccctatccagcgggttatacataatgaattggaacagtactgccgggcccgggccggccgttgcctggaggttggggctcacccgaggtccattaatgacaatcccaatgtcctgcacaggtgctttcttagaccggttggccgagacgtccagcgctggtactctgcccccacccgtggccctgcggccaactgccgccgctccgcgttgcgtggtctccctcccgctgaccgcacttattgctttgatggattctcccgctgtgcttttgctgcagagaccggcgtggccctttactctctgcatgacctttggccagctgatgtcgcagaggctatggcccgccacgggatgacacgcctatatgctgcactacacctccctcctgaggtgctgttgccacccggcacttaccacacaacctcgtatctcctgatccacgacggcgaccgtgccgtcgtaacttatgagggcgatactagtgcaggctacaatcacgatgtttccatacttcgtgcgtggatccgtactactaaaatagttggtgaccacccgttggttatagagcgtgtgcgggccattggatgtcattttgtgctgctgctcaccgcagcccctgagccgtcacctatgccttatgtcccctaccctcgttcaactgaggtgtatgtacgatctatatttggccctggtggctccccatctttgttcccgtcagcctgctctactaaatctacttttcatgctgtcccggttcatatctgggaccggcttatgctttttggtgccaccctggacgatcaggcgttttgttgttcacggctcatgacttacctccgtggtattagctacaaggtcactgtcggtgcgcttgttgctaatgagggatggaatgcctctgaggacgcccttactgcagtgatcactgcggcttacctgactatttgccaccaacgctaccttcgaacccaggcgatatccaagggtatgcgccggttggaggttgagcatgcccagaaattcatcacaaggctctacagctggctatttgagaaatctggtcgtgattatatccccggccgccagcttcagttctatgcacaatgtcggcggtggttatctgcaggcttccacctcgaccccagggtgcttgtcttcgatgaagcagtgccatgccgctgtaggacgtttttgaagaaggtcgcgggtaaattctgctgttttatgcggtggctagggcaggagtgcacctgtttcttggagccagctgagggcctaattggagaccaaggccatgataatgaggcctatgagggttctgaggtcgacccggctgaacctgcacatcttgatgtttcggggacctatgctgtccatgggcatcagcttgaggccctttatagggcactcaatgtcccacatgatattgccgctcgagcctcccggctaacggctactgtcgagcttgttgcaagtccagaccgcttagagtgccgtactgtgcttggtaataagacctttcggacaacggtggttgatggtgcccatcttgaagcaaatggccctgaggagtatgttctatcattcgacgcctctcgtcagtctatgggggccggatcgcacagcctcacatatgagctcacccctgctggtctgcaggtcaggatttcatctaatggcttggattgtaccgccgtattccctcccggcggcgcccctagcgccgcaccgggggaggtggcagccttctgcagcgccctttatagatataacaggttcacccaacggcactcgctaaccggtggattatggttacaccctgaggggttgctgggcatcttcccccctttctctcctggacacatctgggagtctgctaacccattttgtggggaggggaccttgtatacccgaacctggtcaacatctggcttctctagcgacttctccccccctgaggcggccgcccctgttccggctgctgccccggggctgccccaccccaccccacctgttagtgacatttgggtgctgccaccaccctcagaggagtcccagatcgatgcggcacctgtgccccctgtccctaagactgttggattgcctagccccattgtacttgctcctccctcccctcttccttcccccgtgcgtaagccaccatcacccccgccttctcgcactcgtcgtctcctctacacctatcctgacggcgctagggtatatgcggggtcgttgtttgaatcagactgtgactggctagttaacgcctcaaatccgggccaccgtcctggaggtggcctctgccacgccttttaccaacgcttcccagaggcgttttacccaactgaattcattatgcgtgagggccttgcagcatataccctgaccccgcgccctatcattcatgcagtggctcccgactatagggtcgagcagaatccgaagaggcttgaggcagcgtaccgggaaacttgctcccgtcgcggcaccgctgcctatccgcttttgggctcgggtatataccaggtccctgttagtctcagttttgatgcctgggaacgcaatcatcgccccggcgacgagctttacttgactgagcccgctgcagcttggtttgaggctaataagccatcgcagccggcgcttactataactgaggacacggctcgtacggccaatctggcattagagattgatgccgccacagaggttggccgtgcttgtgccggctgcactatcagcccgggggttgtgcattaccagtttactgccggggtcccgggctcgggcaagtcaaggtccatacaacagggagacgtcgatgtggtggttgtgcccacccgggagcttcgtaatagttggcgccgccggggttttgcggctttcacacctcacacagcggcccgtgttactattggtcgccgcgttgtgattgatgaggctccgtccctcccgccgcacttgctgctgctacacatgcaacgggcctcctcggtccatctcctcggcgacccaaatcagattcctgctattgattttgaacatgccggcctggtccccgcgatccgtcccgagcttgcaccaacgagctggtggcatgttacacaccgctgcccggcagatgtgtgtgagcttatacgtggggcctaccctaagatccagaccacgagtcgtgtgctacggtccctgttttggaacgaaccggccattggccagaagctggttttcacgcaggctgctaaggctgctaatcctggtgcgatcacggttcatgaggctcagggtgccaccttcacggagaccacaatcatagccacggctgatgctaggggccttattcagtcatcccgagctcacgctatagtcgcactcacccgccacactgagaagtgtgttattttagatgcccccggcctactgcgcgaggtcggtatttcagatgtgattgtcaataactttttccttgctggtggagaggttggccaccaccgcccctccgtgatacctcgcggtaaccccgatcagaatctcgggactctacaggcattcccgccgtcttgccagattagtgcctaccaccagttggctgaggaattaggccaccgcccagctcctgtcgccgccgtcttacccccttgcccggagcttgagcagggcctgctctacatgccacaagagcttactgtgtccgatagtgtgttggtatttgaactcacagatatagtccattgccgtatggccgctccaagccagcgaaaggctgttctctcaacacttgtcgggaggtatggccgtagaacgaaattatatgaggcggcacattcagatgttcgtgagtccctagctaggttcatccccactatcgggcctgttcaggccaccacatgtgagttgtatgagttggttgaggccatggtggagaagggtcaggacggctctgccgtcctagagcttgacctttgcaatcgtgacgtctcgcgtatcacatttttccaaaaggattgcaataaattcacaactggtgagactattgcccatggcaaggttggccagggtatatcggcctggagtaagaccttctgtgccctgtttggcccgtggttccgcgctatagaaaaagagatattggccctgctcccgcctaatatcttttatggcgacgcttatgaagagtcagtgtttgctgccgctgtgtctggggcggggtcatgtatggtatttgaaaatgatttttcggaatttgacagtactcagaacaacttctctctcggccttgagtgtgtggtcatggaggagtgcggcatgccccagtggttgattaggttgtaccatctggttcggtcagcctggattttgcaggcgccgaaggagtctcttaagggtttttggaagaagcactctggtgagcctggtacccttctctggaacaccgtctggaacatggcgattatagcgcactgttacgagttccgtgactttcgcgttgccgccttcaagggtgatgattcggtggtcctttgcagcgactatcggcagagccgcaatgcggctgccttaattgcaggctgtgggctcaaattgaaggtcgattatcgtcctattgggctgtatgctggggtggtggtggcccctggtttggggacactgcccgacgtggtgcgttttgctggtcggttgtctgaaaagaattggggccccggccctgaacgtgctgagcagctgcgtctcgctgtttgtgatttccttcgagggttgacgaatgttgcgcaggtttgtgttgatgttgtgtcccgtgtttacggagtcagccccgggctggtacataaccttattggcatgctgcagaccattgccgatggcaaggctcacttcacagagaccattaaacctgtgcttgaccttacgaattccatcatacagcgggaagaatgaataacatgtcttttgcatcgcccatgggatcaccatgcgccctagggctgttctgttgttgttcctcgtgcttttgcctatgctgcccgcgccaccggccggtcagccgtctggccgtcgccgtgggcggcgcagcggcggtgccggcggtggtttctggggtgacagggttgattctcagcccttcgccctcccctatattcatccaaccaaccccttcgccgccgatgtcgtttcacaacccggggctggaactcgccctcgacagccgccccgcccccttggctccgcttggcgtgaccagtcccagcgcccctccgctgccccccgccgtcgatctgccccagctggggctgcgccgttgaccgctgtatcaccggctcctgacacagcccctgtgcctgatgttgattcacgcggtgctatcctgcgccggcagtacaatctgtccacgtccccgctcacgtcatctgtcgcctcgggcacaaatctggttctctatgctgccccgcttaatcctctcctgccccttcaggatggcaccaacactcatattatggccactgaggcatccaattatgcccagtatcgggttgttcgagctacgatccgttatcgcccgttggtgccgaatgcagttggcggttatgctatttctatttctttttggcctcaaaccacaactactcccacctctgtcgacatgaattctatcacttccactgatgttaggattttggttcagcccggcattgcctccgagttagtcatccctagtgagcgcctccactaccgcaatcaaggctggcgctctgttgagaccacgggtgtggccgaggaggaggctacttccggtctggtaatgctttgtattcatggctctcctgttaattcctacactaatacaccttatactggtgcactggggctccttgattttgcattagagcttgaatttagaaatctgacacccgggaacacaaacacccgtgtttcccggtataccagcacagcccgtcaccggctgcgccgcggtgctgatgggactgctgagcttaccaccacagcagccacacgtttcatgaaggatttacattttactggcacgaatggtgttggtgaggtgggtcgtggcatcgctctgacattgtttaatctcgctgacacgcttctcggtggtttaccgacagaattgatttcgtcggccgggggtcaactgttttactcccgccctgttgtctcggccaatggcgagccaacagtaaagttatacacatctgttgagaatgcgcagcaagataagggcattaccatcccacacgatatagatctgggtgactcccgtgtggttattcaggattatgataaccagcacgagcaagatcggcctactccgtcacctgccccctcccgccctttctcagttcttcgtgctaatgatgttctgtggctctccctcaccgccgctgagtatgaccagactacgtatgggtcgtccaccaaccctatgtatgtctccgacacagtcacgctcgttaatgtggccactggagcccaggctgtggcccgctctcttgattggtctaaagttaccttggatggccgcccccttactaccattcagcagtattctaagacattctatgtccttccgctccgcgggaagctgtctttctgggaggctggtacgactaaggccggttacccgtataattataatactactgctagtgatcagatcttgattgagaacgcggccggccaccgtgtcgctatttctacctatactactagcttgggtgccggccctacctcgatctctgcggtcggtgtactagctccacattcggccctcgccgttctagaggacaccgttgattaccccgcccgcgctcacacttttgatgatttctgcccggagtgccgtaccctcggtttgcagggttgtgcattccagtctactatcgctgagcttcagcgtcttaaaatgaaggtaggtaaaacccgggagtcttaattaattccttttgtgcccccttcgcagctttctctggctttatttcttatttctgcttttcgcgctccctggaaaaaaaaaaaa

SEQ ID NO: 2 - DNA, 23 bp, Artificial Sequence
  Synthetic Oligonucleotide
aagacauguuauucauuccaccc

SEQ ID NO: 3 - DNA, 56 bp, Artificial Sequence
  Synthetic Oligonucleotide
aagacauguuauucauuccaccctttaaaaaaaaaaaaaaaaaaaaaaaaaaaaaa

SEQ ID NO: 4 - DNA, 23 bp, Artificial Sequence
  Synthetic Oligonucleotide
aagacauguuauucauucywccc

SEQ ID NO: 5 - DNA, 18 bp, Artificial Sequence
  Synthetic Oligonucleotide
tgattgtcagcccttcgc

SEQ ID NO: 6 - DNA, 23 bp, Artificial Sequence
  Synthetic Oligonucleotide
aagacauguuauucauucuaccc

SEQ ID NO: 7 - DNA, 56 bp, Artificial Sequence
  Synthetic Oligonucleotide
aagacauguuauucauucuaccctttaaaaaaaaaaaaaaaaaaaaaaaaaaaaaa

SEQ ID NO: 8 - DNA, 56 bp, Artificial Sequence
  Synthetic Oligonucleotide
aagacauguuauucauucywccctttaaaaaaaaaaaaaaaaaaaaaaaaaaaaaa

SEQ ID NO: 9 - DNA, 50 bp, Artificial Sequence
  Synthetic Oligonucleotide
  promoter (1)..(27)
aatttaatacgactcactatagggagaaggggttggttggatgaatatag

SEQ ID NO: 10 - DNA, 51 bp, Artificial Sequence
  Synthetic Oligonucleotide
  promoter (1)..(27)
aatttaatacgactcactatagggagaaggggttggttggatgaatatagg

SEQ ID NO: 11 - DNA, 52 bp, Artificial Sequence
  Synthetic Oligonucleotide
  promoter (1)..(27)
aatttaatacgactcactatagggagaaggggttggttggatgaatataggg

SEQ ID NO: 12 - DNA, 54 bp, Artificial Sequence
  Synthetic Oligonucleotide
  promoter (1)..(27)
aatttaatacgactcactatagggagaaggggttggttggatgaatatagggga

SEQ ID NO: 13 - DNA, 20 bp, Artificial Sequence
  Synthetic Oligonucleotide
ctatgctgcccgcgccaccg

SEQ ID NO: 14 - DNA, 50 bp, Artificial Sequence
  Synthetic Oligonucleotide
  promoter (1)..(27)
aatttaatacgactcactatagggagaggcgaaggggttggttggatgaa

SEQ ID NO: 15 - DNA, 51 bp, Artificial Sequence
  Synthetic Oligonucleotide
  promoter (1)..(27)
aatttaatacgactcactatagggagagggcgaaggggttggttggatgaa

SEQ ID NO: 16 - DNA, 23 bp, Artificial Sequence
  Synthetic Oligonucleotide
ccggcggtggtttctggggtgac

SEQ ID NO: 17 - DNA, 47 bp, Artificial Sequence
  Synthetic Oligonucleotide
  promoter (1)..(27)
aatttaatacgactcactatagggagaggttggttggatgaatatag

SEQ ID NO: 18 - DNA, 48 bp, Artificial Sequence
  Synthetic Oligonucleotide
  promoter (1)..(27)
aatttaatacgactcactatagggagaggttggttggatgaatatagg

SEQ ID NO: 19 - DNA, 49 bp, Artificial Sequence
  Synthetic Oligonucleotide
  promoter (1)..(27)
aatttaatacgactcactatagggagaggttggttggatgaatataggg

SEQ ID NO: 20 - DNA, 51 bp, Artificial Sequence
  Synthetic Oligonucleotide
  promoter (1)..(27)
aatttaatacgactcactatagggagaggttggttggatgaatatagggga

SEQ ID NO: 21 - DNA, 23 bp, Artificial Sequence
  Synthetic Oligonucleotide
aggggttggttggatgaatatag

SEQ ID NO: 22 - DNA, 24 bp, Artificial Sequence
  Synthetic Oligonucleotide
aggggttggttggatgaatatagg

SEQ ID NO: 23 - DNA, 25 bp, Artificial Sequence
  Synthetic Oligonucleotide
aggggttggttggatgaatataggg

SEQ ID NO: 24 - DNA, 27 bp, Artificial Sequence
  Synthetic Oligonucleotide
aggggttggttggatgaatatagggga

SEQ ID NO: 25 - DNA, 15 bp, Artificial Sequence
  Synthetic Oligonucleotide
ggttggttggatgaa

SEQ ID NO: 26 - DNA, 13 bp, Artificial Sequence
  Synthetic Oligonucleotide
tgctgcccgcgcc

SEQ ID NO: 27 - DNA, 14 bp, Artificial Sequence
  Synthetic Oligonucleotide
cggcggtggtttct

SEQ ID NO: 28 - DNA, 17 bp, Artificial Sequence
  Synthetic Oligonucleotide
  misc_feature (1)..(1): N is c or the residue is absent from the sequence.
  misc_feature (16)..(16): N is g or the residue is absent from the sequence.
  misc_feature (17)..(17): N is g or the residue is absent from the sequence.
ncggcggtggtttctnn

SEQ ID NO: 29 - DNA, 15 bp, Artificial Sequence
  Synthetic Oligonucleotide
ccggcggtggtttct

SEQ ID NO: 30 - DNA, 16 bp, Artificial Sequence
  Synthetic Oligonucleotide
ccggcggtggtttctg

SEQ ID NO: 31 - DNA, 17 bp, Artificial Sequence
  Synthetic Oligonucleotide
ccggcggtggtttctgg

SEQ ID NO: 32 - DNA, 16 bp, Artificial Sequence
  Synthetic Oligonucleotide
cggcggtggtttctgg

SEQ ID NO: 33 - DNA, 16 bp, Artificial Sequence
  Synthetic Oligonucleotide
ctatgctgcccgcgcc

SEQ ID NO: 34 - DNA, 17 bp, Artificial Sequence
  Synthetic Oligonucleotide
ctatgctgcccgcgcca

SEQ ID NO: 35 - DNA, 18 bp, Artificial Sequence
  Synthetic Oligonucleotide
ctatgctgcccgcgccac

SEQ ID NO: 36 - DNA, 16 bp, Artificial Sequence
  Synthetic Oligonucleotide
gaagggctgagaatca

SEQ ID NO: 37 - DNA, 16 bp, Artificial Sequence
  Synthetic Oligonucleotide
gaccggguugauucuc

SEQ ID NO: 38 - DNA, 15 bp, Artificial Sequence
  Synthetic Oligonucleotide
gaccggguugauucu

SEQ ID NO: 39 - DNA, 28 bp, Artificial Sequence
  Synthetic Oligonucleotide
gacagggttgattctcagcccttcgccc

SEQ ID NO: 40 - DNA, 15 bp, Artificial Sequence
  Synthetic Oligonucleotide
gagaatcaacccggt

SEQ ID NO: 41 - DNA, 16 bp, Artificial Sequence
  Synthetic Oligonucleotide
gaccgggttgattctc

SEQ ID NO: 42 - DNA, 21 bp, Artificial Sequence
  Synthetic Oligonucleotide
gaggggcgcugggacuggucg

SEQ ID NO: 43 - DNA, 54 bp, Artificial Sequence
  Synthetic Oligonucleotide
gaggggcgcugggacuggucgtttaaaaaaaaaaaaaaaaaaaaaaaaaaaaaa

SEQ ID NO: 44 - DNA, 92 bp, Artificial Sequence
  Synthetic Oligonucleotide
tgcctatgctgcccgcgccaccggccggtcagccgtctggccgtcgccgtgggcggcgcagcggcggtgccggcggtggtttctggggtgac

SEQ ID NO: 45 - DNA, 23 bp, Artificial Sequence
  Synthetic Oligonucleotide
ggcgaaggggttggttggatgaa

SEQ ID NO: 46 - DNA, 24 bp, Artificial Sequence
  Synthetic Oligonucleotide
gggcgaaggggttggttggatgaa

SEQ ID NO: 47 - DNA, 33 bp, Artificial Sequence
  Synthetic Oligonucleotide
sggcgaaggggttggttggatgaatatagggga

SEQ ID NO: 48 - DNA, 20 bp, Artificial Sequence
  Synthetic Oligonucleotide
ggttggttggatgaatatag

SEQ ID NO: 49 - DNA, 21 bp, Artificial Sequence
  Synthetic Oligonucleotide
ggttggttggatgaatatagg

SEQ ID NO: 50 - DNA, 22 bp, Artificial Sequence
  Synthetic Oligonucleotide
ggttggttggatgaatataggg

SEQ ID NO: 51 - DNA, 24 bp, Artificial Sequence
  Synthetic Oligonucleotide
ggttggttggatgaatatagggga

SEQ ID NO: 52 - DNA, 15 bp, Artificial Sequence
  Synthetic Oligonucleotide
ggtttctggggtgac

SEQ ID NO: 53 - DNA, 16 bp, Artificial Sequence
  Synthetic Oligonucleotide
gtggtttctggggtga

SEQ ID NO: 54 - DNA, 17 bp, Artificial Sequence
  Synthetic Oligonucleotide
gtggtttctggggtgac

SEQ ID NO: 55 - DNA, 22 bp, Artificial Sequence
  Synthetic Oligonucleotide
guugauucucagcccuucgccc

SEQ ID NO: 56 - DNA, 24 bp, Artificial Sequence
  Synthetic Oligonucleotide
sggcgaaggggttggttggatgaa

SEQ ID NO: 57 - DNA, 51 bp, Artificial Sequence
  Synthetic Oligonucleotide
  promoter (1)..(27)
aatttaatacgactcactatagggagasggcgaaggggttggttggatgaa

SEQ ID NO: 58 - DNA, 60 bp, Artificial Sequence
  Synthetic Oligonucleotide
acagggttgattctcagcccttcgccctcccctatattcatccaaccaaccccttcgccs

SEQ ID NO: 59 - DNA, 48 bp, Artificial Sequence
  Synthetic Oligonucleotide
ccggcggtggtttctggggtgacagggttgattctcagcccttcgccc

SEQ ID NO: 60 - DNA, 100 bp, Artificial Sequence
  Synthetic Oligonucleotide
tatgctgcccgcgccaccggccggtcagccgtctggccgtcgccgtgggcggcgcagcggcggtgccggcggtggtttctggggtgacagggttgattct

SEQ ID NO: 61 - DNA, 21 bp, Artificial Sequence
  Synthetic Oligonucleotide
tgcctatgctgcccgcgccac

SEQ ID NO: 62 - DNA, 14 bp, Artificial Sequence
  Synthetic Oligonucleotide
tgctgcccgcgcca

SEQ ID NO: 63 - DNA, 23 bp, Artificial Sequence
  Synthetic Oligonucleotide
tgcctatgctgcccgcgccaccg

SEQ ID NO: 64 - DNA, 15 bp, Artificial Sequence
  Synthetic Oligonucleotide
tgctgcccgcgccac

SEQ ID NO: 65 - DNA, 16 bp, Artificial Sequence
  Synthetic Oligonucleotide
tgctgcccgcgccacc

SEQ ID NO: 66 - DNA, 17 bp, Artificial Sequence
  Synthetic Oligonucleotide
tgctgcccgcgccaccg

SEQ ID NO: 67 - DNA, 18 bp, Artificial Sequence
  Synthetic Oligonucleotide
ugauucucagcccuucgc

SEQ ID NO: 68 - DNA, 25 bp, Artificial Sequence
  Synthetic Oligonucleotide
agggttgattctcagcccttcgccc

SEQ ID NO: 69 - DNA, 94 bp, Artificial Sequence
  Synthetic Oligonucleotide
gccggtcagccgtctggccgtcgccgtgggcggcgcagcggcggtgccggcggtggtttctggggtgacagggttgattctcagcccttcgccc

SEQ ID NO: 70 - DNA, 150 bp, Artificial Sequence
  Synthetic Oligonucleotide
tgcctatgctgcccgcgccaccggccggtcagccgtctggccgtcgccgtgggcggcgcagcggcggtgccggcggtggtttctggggtgacagggttgattctcagcccttcgccctcccctatattcatccaaccaaccccttcgccg

SEQ ID NO: 71 - DNA, 18 bp, Artificial Sequence
  Synthetic Oligonucleotide
ugauugucagcccuucgc

SEQ ID NO: 72 - DNA, 17 bp, Artificial Sequence
  Synthetic Oligonucleotide
ugauugucagcccuucg

SEQ ID NO: 73 - DNA, 27 bp, Artificial Sequence
  Synthetic Oligonucleotide
  promoter (1)..(27)
aatttaatacgactcactatagggaga

SEQ ID NO: 74 - DNA, 57 bp, Artificial Sequence
  Synthetic Oligonucleotide
accgccgcugcgccgcccacggcgtttaaaaaaaaaaaaaaaaaaaaaaaaaaaaaa

SEQ ID NO: 75 - DNA, 24 bp, Artificial Sequence
  Synthetic Oligonucleotide
accgccgcugcgccgcccacggcg

SEQ ID NO: 76 - DNA, 57 bp, Artificial Sequence
  Synthetic Oligonucleotide
agcggcggggcgcugggccugguctttaaaaaaaaaaaaaaaaaaaaaaaaaaaaaa

SEQ ID NO: 77 - DNA, 24 bp, Artificial Sequence
  Synthetic Oligonucleotide
agcggcggggcgcugggccugguc

SEQ ID NO: 78 - DNA, 24 bp, Artificial Sequence
  Synthetic Oligonucleotide
ccacaagcuuagaagauagagagg

SEQ ID NO: 79 - DNA, 16 bp, Artificial Sequence
  Synthetic Oligonucleotide
ctatcttctaagcttg